European Patent Specification EP 3 363 818 B1, published June 25, 2025. Title: Method to generate CH3 domain mutant pairs of heterodimeric Fc using yeast mating and CH3 domain mutant pairs thereby. Applicant: AJOU UNIVERSITY INDUSTRY-ACADEMIC COOPERATION FOUNDATION. The sequence listing filed with the application follows.

SEQUENCE LISTING (100 sequences)

SEQ ID NO: 1 - protein, 107 aa, Artificial Sequence
  Wild type CH3A
GQPREPQVYTLPPSRDELTKNQVSLTCLVKGFYPSDIAVEWESNGQPENNYKTTPPVLDSDGSFFLYSKLTVDKSRWQQGNVFSCSVMHEALHNHYTQKSLSLSPGK

SEQ ID NO: 2 - protein, 107 aa, Artificial Sequence
  W-VT CH3A
GQPREPQVYTLPPSRDELTKNQVSLTCLVKGFYPSDIAVEWESNGQPENNYKTTPPVLDSDGSFFLYSWLTVDKSRWQQGNVFSCSVMHEALHNHYTQKSLSLSPGK

SEQ ID NO: 3 - protein, 107 aa, Artificial Sequence
  W-VT CH3B
GQPREPQVYTLPPSRDELTKNQVSLTCLVKGFYPSDIAVEWESNGQPENNYKTTPPVLVSDGSFTLYSKLTVDKSRWQQGNVFSCSVMHEALHNHYTQKSLSLSPGK

SEQ ID NO: 4 - protein, 107 aa, Artificial Sequence
  EW-RVT CH3A
GQPREPQVYTLPPSRDELTENQVSLTCLVKGFYPSDIAVEWESNGQPENNYKTTPPVLDSDGSFFLYSWLTVDKSRWQQGNVFSCSVMHEALHNHYTQKSLSLSPGK

SEQ ID NO: 5 - protein, 107 aa, Artificial Sequence
  EW-RVT CH3B
GQPREPRVYTLPPSRDELTKNQVSLTCLVKGFYPSDIAVEWESNGQPENNYKTTPPVLVSDGSFTLYSKLTVDKSRWQQGNVFSCSVMHEALHNHYTQKSLSLSPGK

SEQ ID NO: 6 - protein, 107 aa, Artificial Sequence
  A107 CH3A
GQPREPQVYTLPPSRDELTKNQVSLTCLVEGFYPSDIAVEWESNGQPENNYKTTPPVLDSDGSFFLYSWLTVDKSRWQQGNVFSCSVMHEALHNHYTQKSLSLSPGK

SEQ ID NO: 7 - protein, 107 aa, Artificial Sequence
  A107 CH3B
GQPREPQVYTLPPSRDNLTKNQVSLTCLVKGFYPSDIAVEWESNGQPENNYKTTPPVLVSDGSFTLYSKLTVDKSRWQQGNVFSCSVMHEALHNHYTQKSLSLSPGK

SEQ ID NO: 8 - protein, 107 aa, Artificial Sequence; identical to SEQ ID NO: 6
  A108 CH3A

SEQ ID NO: 9 - protein, 107 aa, Artificial Sequence
  A108 CH3B
GQPREPQVYTLPPSRDILTKNQVTLTCLVKGFYPSDIAVEWESNGQPENNYKTTPPVLVSDGSFTLYSKLTVDKSRWQQGNVFSCSVMHEALHNHYTQKSLSLSPGK

SEQ ID NO: 10 - protein, 107 aa, Artificial Sequence
  A109 CH3A
GQPREPQVYTLPPSRDELTKNQVSLTCLVMGFYPSDIAVEWESNGQPENNYKTTPPVLDSDGSFFLYSWLTVDKSRWQQGNVFSCSVMHEALHNHYTQKSLSLSPGK

SEQ ID NO: 11 - protein, 107 aa, Artificial Sequence
  A109 CH3B
GQPREPQVYTLPPSRDMLTKNQVWLTCLVKGFYPSDIAVEWESNGQPENNYKTTPPVLVSDGSFTLYSKLTVDKSRWQQGNVFSCSVMHEALHNHYTQKSLSLSPGK

SEQ ID NO: 12 - protein, 107 aa, Artificial Sequence
  A146 CH3A
GQPREPQVYTLPPSRDELTKNQVSLTCLVDGFYPSDIAVEWESNGQPENNYKTTPPVLDSDGSFFLYSWLTVDKSRWQQGNVFSCSVMHEALHNHYTQKSLSLSPGK

SEQ ID NO: 13 - protein, 107 aa, Artificial Sequence
  A146 CH3B
GQPREPQVYTLPPSRDMLTKNQVSLTCLVKGFYPSDIAVEWESNGQPENNYKTTPPVLVSDGSFTLYSKLTVDKSRWQQGNVFSCSVMHEALHNHYTQKSLSLSPGK

SEQ ID NO: 14 - protein, 107 aa, Artificial Sequence
  B121 CH3A
GQPREPQVYTLPPSRDELTKNQVSLTCLVKGFYPSDIAVEWESNGQPENNYKTTPPVLESDGSFFLYSWLTVDKSRWQQGNVFSCSVMHEALHNHYTQKSLSLSPGK

SEQ ID NO: 15 - protein, 107 aa, Artificial Sequence
  B121 CH3B
GQPREPQVYTLPPSRDELTKNQVSLTCLVKGFYPSDIAVEWESNGQPENNYETTPPVLVSDGSFTLYSKLTVDKSRWQQGNVFSCSVMHEALHNHYTQKSLSLSPGK

SEQ ID NO: 16 - protein, 107 aa, Artificial Sequence
  B135 CH3A
GQPREPQVYTLPPSRDELTKNQVSLTCLVKGFYPSDIAVEWESNGQPENNYKTTPPVLLSDGSFFLYSWLTVDKSRWQQGNVFSCSVMHEALHNHYTQKSLSLSPGK

SEQ ID NO: 17 - protein, 107 aa, Artificial Sequence
  B135 CH3B
GQPREPQVYTLPPSRDELTKNQVSLTCLVKGFYPSDIAVEWESNGQPENNYSTTPPVLVSDGSFTLYSLLTVDKSRWQQGNVFSCSVMHEALHNHYTQKSLSLSPGK

SEQ ID NO: 18 - protein, 107 aa, Artificial Sequence; identical to SEQ ID NO: 16
  B168 CH3A

SEQ ID NO: 19 - protein, 107 aa, Artificial Sequence
  B168 CH3B
GQPREPQVYTLPPSRDELTKNQVSLTCLVKGFYPSDIAVEWESNGQPENNYGTTPPVLVSDGSFTLYSMLTVDKSRWQQGNVFSCSVMHEALHNHYTQKSLSLSPGK

SEQ ID NO: 20 - protein, 107 aa, Artificial Sequence
  A205 CH3A
GQPREPQVYTLPPSRDDLTKNQVWLTCLVEGFYPSDIAVEWESNGQPENNYKTTPPVLDSDGSFFLYSKLTVDKSRWQQGNVFSCSVMHEALHNHYTQKSLSLSPGK

SEQ ID NO: 21 - protein, 107 aa, Artificial Sequence
  A205 CH3B
GQPREPQVYTLPPSRDNLTKNQVSLTCLVRGFYPSDIAVEWESNGQPENNYKTTPPVLDSDGSFFLYSKLTVDKSRWQQGNVFSCSVMHEALHNHYTQKSLSLSPGK

SEQ ID NO: 22 - protein, 107 aa, Artificial Sequence
  A210 CH3A
GQPREPQVYTLPPSRDALTKNQVYLTCLVEGFYPSDIAVEWESNGQPENNYKTTPPVLDSDGSFFLYSKLTVDKSRWQQGNVFSCSVMHEALHNHYTQKSLSLSPGK

SEQ ID NO: 23 - protein, 107 aa, Artificial Sequence
  A210 CH3B
GQPREPQVYTLPPSRDNLTKNQVSLTCLVHGFYPSDIAVEWESNGQPENNYKTTPPVLDSDGSFFLYSKLTVDKSRWQQGNVFSCSVMHEALHNHYTQKSLSLSPGK

SEQ ID NO: 24 - protein, 107 aa, Artificial Sequence
  A216 CH3A
GQPREPQVYTLPPSRDGLTKNQVWLTCLVEGFYPSDIAVEWESNGQPENNYKTTPPVLDSDGSFFLYSKLTVDKSRWQQGNVFSCSVMHEALHNHYTQKSLSLSPGK

SEQ ID NO: 25 - protein, 107 aa, Artificial Sequence
  A216 CH3B
GQPREPQVYTLPPSRDNLTKNQVSLTCLVKGFYPSDIAVEWESNGQPENNYKTTPPVLDSDGSFFLYSKLTVDKSRWQQGNVFSCSVMHEALHNHYTQKSLSLSPGK

SEQ ID NO: 26 - protein, 107 aa, Artificial Sequence
  A241 CH3A
GQPREPQVYTLPPSRDNLTKNQVWLTCLVEGFYPSDIAVEWESNGQPENNYKTTPPVLDSDGSFFLYSKLTVDKSRWQQGNVFSCSVMHEALHNHYTQKSLSLSPGK

SEQ ID NO: 27 - protein, 107 aa, Artificial Sequence; identical to SEQ ID NO: 25
  A241 CH3B

SEQ ID NO: 28 - protein, 107 aa, Artificial Sequence
  B212 CH3A
GQPREPQVYTLPPSRDELTKNQVSLTCLVKGFYPSDIAVEWESNGQPENNYITTPPVLLSDGSFFLYSKLTVDKSRWQQGNVFSCSVMHEALHNHYTQKSLSLSPGK

SEQ ID NO: 29 - protein, 107 aa, Artificial Sequence
  B212 CH3B
GQPREPQVYTLPPSRDELTKNQVSLTCLVKGFYPSDIAVEWESNGQPENNYGTTPPVLGSDGSFFLYSMLTVDKSRWQQGNVFSCSVMHEALHNHYTQKSLSLSPGK

SEQ ID NO: 30 - protein, 107 aa, Artificial Sequence
  B215 CH3A
GQPREPQVYTLPPSRDELTKNQVSLTCLVKGFYPSDIAVEWESNGQPENNYRTTPPVLLSDGSFFLYSRLTVDKSRWQQGNVFSCSVMHEALHNHYTQKSLSLSPGK

SEQ ID NO: 31 - protein, 107 aa, Artificial Sequence
  B215 CH3B
GQPREPQVYTLPPSRDELTKNQVSLTCLVKGFYPSDIAVEWESNGQPENNYGTTPPVLWSDGSFFLYSMLTVDKSRWQQGNVFSCSVMHEALHNHYTQKSLSLSPGK

SEQ ID NO: 32 - protein, 107 aa, Artificial Sequence
  B235 CH3A
GQPREPQVYTLPPSRDELTKNQVSLTCLVKGFYPSDIAVEWESNGQPENNYCTTPPVLLSDGSFFLYSKLTVDKSRWQQGNVFSCSVMHEALHNHYTQKSLSLSPGK

SEQ ID NO: 33 - protein, 107 aa, Artificial Sequence
  B235 CH3B
GQPREPQVYTLPPSRDELTKNQVSLTCLVKGFYPSDIAVEWESNGQPENNYGTTPPVLCSDGSFFLYSMLTVDKSRWQQGNVFSCSVMHEALHNHYTQKSLSLSPGK

SEQ ID NO: 34 - protein, 223 aa, Artificial Sequence
  B239 CH3A
TCPPCPAPELLGGPSVFLFPPKPKDTLMISRTPEVTCVVVDVSHEDPEVKFNWYVDGVEVHNAKTKPREEQYNSTYRVVSVLTVLHQDWLNGKEYKCKVSNKALPAPIEKTISKAKGQPREPQVYTLPPSRDELTKNQVSLTCLVKGFYPSDIAVEWESNGQPENNYLTTPPVLLSDGSFFLYSKLTVDKSRWQQGNVFSCSVMHEALHNHYTQKSLSLSPGK

SEQ ID NO: 35 - protein, 223 aa, Artificial Sequence
  B239 CH3B
TCPPCPAPELLGGPSVFLFPPKPKDTLMISRTPEVTCVVVDVSHEDPEVKFNWYVDGVEVHNAKTKPREEQYNSTYRVVSVLTVLHQDWLNGKEYKCKVSNKALPAPIEKTISKAKGQPREPQVYTLPPSRDELTKNQVSLTCLVKGFYPSDIAVEWESNGQPENNYGTTPPVLSSDGSFFLYSMLTVDKSRWQQGNVFSCSVMHEALHNHYTQKSLSLSPGK

SEQ ID NO: 36 - protein, 107 aa, Artificial Sequence
  B240 CH3A
GQPREPQVYTLPPSRDELTKNQVSLTCLVKGFYPSDIAVEWESNGQPENNYSTTPPVLLSDGSFFLYSRLTVDKSRWQQGNVFSCSVMHEALHNHYTQKSLSLSPGK

SEQ ID NO: 37 - protein, 107 aa, Artificial Sequence; identical to SEQ ID NO: 29
  B240 CH3B

SEQ ID NO: 38 - protein, 107 aa, Artificial Sequence
  B256 CH3A
GQPREPQVYTLPPSRDELTKNQVSLTCLVKGFYPSDIAVEWESNGQPENNYNTTPPVLLSDGSFFLYSKLTVDKSRWQQGNVFSCSVMHEALHNHYTQKSLSLSPGK

SEQ ID NO: 39 - protein, 107 aa, Artificial Sequence
  B256 CH3B
GQPREPQVYTLPPSRDELTKNQVSLTCLVKGFYPSDIAVEWESNGQPENNYGTTPPVLVSDGSFFLYSMLTVDKSRWQQGNVFSCSVMHEALHNHYTQKSLSLSPGK

SEQ ID NO: 40 - protein, 107 aa, Artificial Sequence
  A107w/oW-VT CH3A
GQPREPQVYTLPPSRDELTKNQVSLTCLVEGFYPSDIAVEWESNGQPENNYKTTPPVLDSDGSFFLYSKLTVDKSRWQQGNVFSCSVMHEALHNHYTQKSLSLSPGK

SEQ ID NO: 41 - protein, 107 aa, Artificial Sequence; identical to SEQ ID NO: 25
  A107w/oW-VT CH3B

SEQ ID NO: 42 - protein, 107 aa, Artificial Sequence
  A109w/oW-VT CH3A
GQPREPQVYTLPPSRDELTKNQVSLTCLVMGFYPSDIAVEWESNGQPENNYKTTPPVLDSDGSFFLYSKLTVDKSRWQQGNVFSCSVMHEALHNHYTQKSLSLSPGK

SEQ ID NO: 43 - protein, 107 aa, Artificial Sequence
  A109w/oW-VT CH3B
GQPREPQVYTLPPSRDMLTKNQVWLTCLVKGFYPSDIAVEWESNGQPENNYKTTPPVLDSDGSFFLYSKLTVDKSRWQQGNVFSCSVMHEALHNHYTQKSLSLSPGK

SEQ ID NO: 44 - protein, 107 aa, Artificial Sequence
  A146w/oW-VT CH3A
GQPREPQVYTLPPSRDELTKNQVSLTCLVDGFYPSDIAVEWESNGQPENNYKTTPPVLDSDGSFFLYSKLTVDKSRWQQGNVFSCSVMHEALHNHYTQKSLSLSPGK

SEQ ID NO: 45 - protein, 107 aa, Artificial Sequence
  A146w/oW-VT CH3B
GQPREPQVYTLPPSRDMLTKNQVSLTCLVKGFYPSDIAVEWESNGQPENNYKTTPPVLDSDGSFFLYSKLTVDKSRWQQGNVFSCSVMHEALHNHYTQKSLSLSPGK

SEQ ID NO: 46 - protein, 107 aa, Artificial Sequence
  B168w/oW-VT CH3A
GQPREPQVYTLPPSRDELTKNQVSLTCLVKGFYPSDIAVEWESNGQPENNYKTTPPVLLSDGSFFLYSKLTVDKSRWQQGNVFSCSVMHEALHNHYTQKSLSLSPGK

SEQ ID NO: 47 - protein, 107 aa, Artificial Sequence
  B168w/oW-VT CH3B
GQPREPQVYTLPPSRDELTKNQVSLTCLVKGFYPSDIAVEWESNGQPENNYGTTPPVLDSDGSFFLYSMLTVDKSRWQQGNVFSCSVMHEALHNHYTQKSLSLSPGK

SEQ ID NO: 48 - protein, 107 aa, Artificial Sequence
  KiH (Genentech) CH3A
GQPREPQVYTLPPSRDELTKNQVSLSCAVKGFYPSDIAVEWESNGQPENNYKTTPPVLDSDGSFFLVSKLTVDKSRWQQGNVFSCSVMHEALHNHYTQKSLSLSPGK

SEQ ID NO: 49 - protein, 107 aa, Artificial Sequence
  KiH (Genentech) CH3B
GQPREPQVYTLPPSRDELTKNQVSLWCLVKGFYPSDIAVEWESNGQPENNYKTTPPVLDSDGSFFLYSKLTVDKSRWQQGNVFSCSVMHEALHNHYTQKSLSLSPGK

SEQ ID NO: 50 - protein, 107 aa, Artificial Sequence; identical to SEQ ID NO: 48
  Hole-Hole (Genentech) CH3A

SEQ ID NO: 51 - protein, 223 aa, Artificial Sequence
  Wild type Fc (CH3A included)
TCPPCPAPELLGGPSVFLFPPKPKDTLMISRTPEVTCVVVDVSHEDPEVKFNWYVDGVEVHNAKTKPREEQYNSTYRVVSVLTVLHQDWLNGKEYKCKVSNKALPAPIEKTISKAKGQPREPQVYTLPPSRDELTKNQVSLTCLVKGFYPSDIAVEWESNGQPENNYKTTPPVLDSDGSFFLYSKLTVDKSRWQQGNVFSCSVMHEALHNHYTQKSLSLSPGK

SEQ ID NO: 52 - protein, 223 aa, Artificial Sequence
  W-VT Fc (CH3A included)
TCPPCPAPELLGGPSVFLFPPKPKDTLMISRTPEVTCVVVDVSHEDPEVKFNWYVDGVEVHNAKTKPREEQYNSTYRVVSVLTVLHQDWLNGKEYKCKVSNKALPAPIEKTISKAKGQPREPQVYTLPPSRDELTKNQVSLTCLVKGFYPSDIAVEWESNGQPENNYKTTPPVLDSDGSFFLYSWLTVDKSRWQQGNVFSCSVMHEALHNHYTQKSLSLSPGK

SEQ ID NO: 53 - protein, 223 aa, Artificial Sequence
  W-VT Fc (CH3B included)
TCPPCPAPELLGGPSVFLFPPKPKDTLMISRTPEVTCVVVDVSHEDPEVKFNWYVDGVEVHNAKTKPREEQYNSTYRVVSVLTVLHQDWLNGKEYKCKVSNKALPAPIEKTISKAKGQPREPQVYTLPPSRDELTKNQVSLTCLVKGFYPSDIAVEWESNGQPENNYKTTPPVLVSDGSFTLYSKLTVDKSRWQQGNVFSCSVMHEALHNHYTQKSLSLSPGK

SEQ ID NO: 54 - protein, 223 aa, Artificial Sequence
  EW-RVT Fc (CH3A included)
TCPPCPAPELLGGPSVFLFPPKPKDTLMISRTPEVTCVVVDVSHEDPEVKFNWYVDGVEVHNAKTKPREEQYNSTYRVVSVLTVLHQDWLNGKEYKCKVSNKALPAPIEKTISKAKGQPREPQVYTLPPSRDELTENQVSLTCLVKGFYPSDIAVEWESNGQPENNYKTTPPVLDSDGSFFLYSWLTVDKSRWQQGNVFSCSVMHEALHNHYTQKSLSLSPGK

SEQ ID NO: 55 - protein, 223 aa, Artificial Sequence
  EW-RVT Fc (CH3B included)
TCPPCPAPELLGGPSVFLFPPKPKDTLMISRTPEVTCVVVDVSHEDPEVKFNWYVDGVEVHNAKTKPREEQYNSTYRVVSVLTVLHQDWLNGKEYKCKVSNKALPAPIEKTISKAKGQPREPRVYTLPPSRDELTKNQVSLTCLVKGFYPSDIAVEWESNGQPENNYKTTPPVLVSDGSFTLYSKLTVDKSRWQQGNVFSCSVMHEALHNHYTQKSLSLSPGK

SEQ ID NO: 56 - protein, 223 aa, Artificial Sequence
  A107 Fc (CH3A included)
TCPPCPAPELLGGPSVFLFPPKPKDTLMISRTPEVTCVVVDVSHEDPEVKFNWYVDGVEVHNAKTKPREEQYNSTYRVVSVLTVLHQDWLNGKEYKCKVSNKALPAPIEKTISKAKGQPREPQVYTLPPSRDELTKNQVSLTCLVEGFYPSDIAVEWESNGQPENNYKTTPPVLDSDGSFFLYSWLTVDKSRWQQGNVFSCSVMHEALHNHYTQKSLSLSPGK

SEQ ID NO: 57 - protein, 223 aa, Artificial Sequence
  A107 Fc (CH3B included)
TCPPCPAPELLGGPSVFLFPPKPKDTLMISRTPEVTCVVVDVSHEDPEVKFNWYVDGVEVHNAKTKPREEQYNSTYRVVSVLTVLHQDWLNGKEYKCKVSNKALPAPIEKTISKAKGQPREPQVYTLPPSRDNLTKNQVSLTCLVKGFYPSDIAVEWESNGQPENNYKTTPPVLVSDGSFTLYSKLTVDKSRWQQGNVFSCSVMHEALHNHYTQKSLSLSPGK

SEQ ID NO: 58 - protein, 223 aa, Artificial Sequence; identical to SEQ ID NO: 56
  A108 Fc (CH3A included)

SEQ ID NO: 59 - protein, 223 aa, Artificial Sequence
  A108 Fc (CH3B included)
TCPPCPAPELLGGPSVFLFPPKPKDTLMISRTPEVTCVVVDVSHEDPEVKFNWYVDGVEVHNAKTKPREEQYNSTYRVVSVLTVLHQDWLNGKEYKCKVSNKALPAPIEKTISKAKGQPREPQVYTLPPSRDILTKNQVTLTCLVKGFYPSDIAVEWESNGQPENNYKTTPPVLVSDGSFTLYSKLTVDKSRWQQGNVFSCSVMHEALHNHYTQKSLSLSPGK

SEQ ID NO: 60 - protein, 223 aa, Artificial Sequence
  A109 Fc (CH3A included)
TCPPCPAPELLGGPSVFLFPPKPKDTLMISRTPEVTCVVVDVSHEDPEVKFNWYVDGVEVHNAKTKPREEQYNSTYRVVSVLTVLHQDWLNGKEYKCKVSNKALPAPIEKTISKAKGQPREPQVYTLPPSRDELTKNQVSLTCLVMGFYPSDIAVEWESNGQPENNYKTTPPVLDSDGSFFLYSWLTVDKSRWQQGNVFSCSVMHEALHNHYTQKSLSLSPGK

SEQ ID NO: 61 - protein, 223 aa, Artificial Sequence
  A109 Fc (CH3B included)
TCPPCPAPELLGGPSVFLFPPKPKDTLMISRTPEVTCVVVDVSHEDPEVKFNWYVDGVEVHNAKTKPREEQYNSTYRVVSVLTVLHQDWLNGKEYKCKVSNKALPAPIEKTISKAKGQPREPQVYTLPPSRDMLTKNQVWLTCLVKGFYPSDIAVEWESNGQPENNYKTTPPVLVSDGSFTLYSKLTVDKSRWQQGNVFSCSVMHEALHNHYTQKSLSLSPGK

SEQ ID NO: 62 - protein, 223 aa, Artificial Sequence
  A146 Fc (CH3A included)
TCPPCPAPELLGGPSVFLFPPKPKDTLMISRTPEVTCVVVDVSHEDPEVKFNWYVDGVEVHNAKTKPREEQYNSTYRVVSVLTVLHQDWLNGKEYKCKVSNKALPAPIEKTISKAKGQPREPQVYTLPPSRDELTKNQVSLTCLVDGFYPSDIAVEWESNGQPENNYKTTPPVLDSDGSFFLYSWLTVDKSRWQQGNVFSCSVMHEALHNHYTQKSLSLSPGK

SEQ ID NO: 63 - protein, 223 aa, Artificial Sequence
  A146 Fc (CH3B included)
TCPPCPAPELLGGPSVFLFPPKPKDTLMISRTPEVTCVVVDVSHEDPEVKFNWYVDGVEVHNAKTKPREEQYNSTYRVVSVLTVLHQDWLNGKEYKCKVSNKALPAPIEKTISKAKGQPREPQVYTLPPSRDMLTKNQVSLTCLVKGFYPSDIAVEWESNGQPENNYKTTPPVLVSDGSFTLYSKLTVDKSRWQQGNVFSCSVMHEALHNHYTQKSLSLSPGK

SEQ ID NO: 64 - protein, 223 aa, Artificial Sequence
  B121 Fc (CH3A included)
TCPPCPAPELLGGPSVFLFPPKPKDTLMISRTPEVTCVVVDVSHEDPEVKFNWYVDGVEVHNAKTKPREEQYNSTYRVVSVLTVLHQDWLNGKEYKCKVSNKALPAPIEKTISKAKGQPREPQVYTLPPSRDELTKNQVSLTCLVKGFYPSDIAVEWESNGQPENNYKTTPPVLESDGSFFLYSWLTVDKSRWQQGNVFSCSVMHEALHNHYTQKSLSLSPGK

SEQ ID NO: 65 - protein, 223 aa, Artificial Sequence
  B121 Fc (CH3B included)
TCPPCPAPELLGGPSVFLFPPKPKDTLMISRTPEVTCVVVDVSHEDPEVKFNWYVDGVEVHNAKTKPREEQYNSTYRVVSVLTVLHQDWLNGKEYKCKVSNKALPAPIEKTISKAKGQPREPQVYTLPPSRDELTKNQVSLTCLVKGFYPSDIAVEWESNGQPENNYETTPPVLVSDGSFTLYSKLTVDKSRWQQGNVFSCSVMHEALHNHYTQKSLSLSPGK

SEQ ID NO: 66 - protein, 223 aa, Artificial Sequence
  B135 Fc (CH3A included)
TCPPCPAPELLGGPSVFLFPPKPKDTLMISRTPEVTCVVVDVSHEDPEVKFNWYVDGVEVHNAKTKPREEQYNSTYRVVSVLTVLHQDWLNGKEYKCKVSNKALPAPIEKTISKAKGQPREPQVYTLPPSRDELTKNQVSLTCLVKGFYPSDIAVEWESNGQPENNYKTTPPVLLSDGSFFLYSWLTVDKSRWQQGNVFSCSVMHEALHNHYTQKSLSLSPGK

SEQ ID NO: 67 - protein, 223 aa, Artificial Sequence
  B135 Fc (CH3B included)
TCPPCPAPELLGGPSVFLFPPKPKDTLMISRTPEVTCVVVDVSHEDPEVKFNWYVDGVEVHNAKTKPREEQYNSTYRVVSVLTVLHQDWLNGKEYKCKVSNKALPAPIEKTISKAKGQPREPQVYTLPPSRDELTKNQVSLTCLVKGFYPSDIAVEWESNGQPENNYSTTPPVLVSDGSFTLYSLLTVDKSRWQQGNVFSCSVMHEALHNHYTQKSLSLSPGK

SEQ ID NO: 68 - protein, 223 aa, Artificial Sequence; identical to SEQ ID NO: 66
  B168 Fc (CH3A included)

SEQ ID NO: 69 - protein, 223 aa, Artificial Sequence
  B168 Fc (CH3B included)
TCPPCPAPELLGGPSVFLFPPKPKDTLMISRTPEVTCVVVDVSHEDPEVKFNWYVDGVEVHNAKTKPREEQYNSTYRVVSVLTVLHQDWLNGKEYKCKVSNKALPAPIEKTISKAKGQPREPQVYTLPPSRDELTKNQVSLTCLVKGFYPSDIAVEWESNGQPENNYGTTPPVLVSDGSFTLYSMLTVDKSRWQQGNVFSCSVMHEALHNHYTQKSLSLSPGK

SEQ ID NO: 70 - protein, 223 aa, Artificial Sequence
  A205 Fc (CH3A included)
TCPPCPAPELLGGPSVFLFPPKPKDTLMISRTPEVTCVVVDVSHEDPEVKFNWYVDGVEVHNAKTKPREEQYNSTYRVVSVLTVLHQDWLNGKEYKCKVSNKALPAPIEKTISKAKGQPREPQVYTLPPSRDDLTKNQVWLTCLVEGFYPSDIAVEWESNGQPENNYKTTPPVLDSDGSFFLYSKLTVDKSRWQQGNVFSCSVMHEALHNHYTQKSLSLSPGK

SEQ ID NO: 71 - protein, 223 aa, Artificial Sequence
  A205 Fc (CH3 included)
TCPPCPAPELLGGPSVFLFPPKPKDTLMISRTPEVTCVVVDVSHEDPEVKFNWYVDGVEVHNAKTKPREEQYNSTYRVVSVLTVLHQDWLNGKEYKCKVSNKALPAPIEKTISKAKGQPREPQVYTLPPSRDNLTKNQVSLTCLVRGFYPSDIAVEWESNGQPENNYKTTPPVLDSDGSFFLYSKLTVDKSRWQQGNVFSCSVMHEALHNHYTQKSLSLSPGK

SEQ ID NO: 72 - protein, 223 aa, Artificial Sequence
  A210 Fc (CH3A included)
TCPPCPAPELLGGPSVFLFPPKPKDTLMISRTPEVTCVVVDVSHEDPEVKFNWYVDGVEVHNAKTKPREEQYNSTYRVVSVLTVLHQDWLNGKEYKCKVSNKALPAPIEKTISKAKGQPREPQVYTLPPSRDALTKNQVYLTCLVEGFYPSDIAVEWESNGQPENNYKTTPPVLDSDGSFFLYSKLTVDKSRWQQGNVFSCSVMHEALHNHYTQKSLSLSPGK

SEQ ID NO: 73 - protein, 223 aa, Artificial Sequence
  A210 Fc (CH3B included)
TCPPCPAPELLGGPSVFLFPPKPKDTLMISRTPEVTCVVVDVSHEDPEVKFNWYVDGVEVHNAKTKPREEQYNSTYRVVSVLTVLHQDWLNGKEYKCKVSNKALPAPIEKTISKAKGQPREPQVYTLPPSRDNLTKNQVSLTCLVHGFYPSDIAVEWESNGQPENNYKTTPPVLDSDGSFFLYSKLTVDKSRWQQGNVFSCSVMHEALHNHYTQKSLSLSPGK

SEQ ID NO: 74 - protein, 223 aa, Artificial Sequence
  A216 Fc (CH3A included)
TCPPCPAPELLGGPSVFLFPPKPKDTLMISRTPEVTCVVVDVSHEDPEVKFNWYVDGVEVHNAKTKPREEQYNSTYRVVSVLTVLHQDWLNGKEYKCKVSNKALPAPIEKTISKAKGQPREPQVYTLPPSRDGLTKNQVWLTCLVEGFYPSDIAVEWESNGQPENNYKTTPPVLDSDGSFFLYSKLTVDKSRWQQGNVFSCSVMHEALHNHYTQKSLSLSPGK

SEQ ID NO: 75 - protein, 223 aa, Artificial Sequence
  A216 Fc (CH3B included)
TCPPCPAPELLGGPSVFLFPPKPKDTLMISRTPEVTCVVVDVSHEDPEVKFNWYVDGVEVHNAKTKPREEQYNSTYRVVSVLTVLHQDWLNGKEYKCKVSNKALPAPIEKTISKAKGQPREPQVYTLPPSRDNLTKNQVSLTCLVKGFYPSDIAVEWESNGQPENNYKTTPPVLDSDGSFFLYSKLTVDKSRWQQGNVFSCSVMHEALHNHYTQKSLSLSPGK

SEQ ID NO: 76 - protein, 223 aa, Artificial Sequence
  A241 Fc (CH3A included)
TCPPCPAPELLGGPSVFLFPPKPKDTLMISRTPEVTCVVVDVSHEDPEVKFNWYVDGVEVHNAKTKPREEQYNSTYRVVSVLTVLHQDWLNGKEYKCKVSNKALPAPIEKTISKAKGQPREPQVYTLPPSRDNLTKNQVWLTCLVEGFYPSDIAVEWESNGQPENNYKTTPPVLDSDGSFFLYSKLTVDKSRWQQGNVFSCSVMHEALHNHYTQKSLSLSPGK

SEQ ID NO: 77 - protein, 223 aa, Artificial Sequence; identical to SEQ ID NO: 75
  A241 Fc (CH3B included)

SEQ ID NO: 78 - protein, 223 aa, Artificial Sequence
  B212 Fc (CH3A included)
TCPPCPAPELLGGPSVFLFPPKPKDTLMISRTPEVTCVVVDVSHEDPEVKFNWYVDGVEVHNAKTKPREEQYNSTYRVVSVLTVLHQDWLNGKEYKCKVSNKALPAPIEKTISKAKGQPREPQVYTLPPSRDELTKNQVSLTCLVKGFYPSDIAVEWESNGQPENNYITTPPVLLSDGSFFLYSKLTVDKSRWQQGNVFSCSVMHEALHNHYTQKSLSLSPGK

SEQ ID NO: 79 - protein, 223 aa, Artificial Sequence
  B212 Fc (CH3B included)
TCPPCPAPELLGGPSVFLFPPKPKDTLMISRTPEVTCVVVDVSHEDPEVKFNWYVDGVEVHNAKTKPREEQYNSTYRVVSVLTVLHQDWLNGKEYKCKVSNKALPAPIEKTISKAKGQPREPQVYTLPPSRDELTKNQVSLTCLVKGFYPSDIAVEWESNGQPENNYGTTPPVLGSDGSFFLYSMLTVDKSRWQQGNVFSCSVMHEALHNHYTQKSLSLSPGK

SEQ ID NO: 80 - protein, 223 aa, Artificial Sequence
  B215 Fc (CH3A included)
TCPPCPAPELLGGPSVFLFPPKPKDTLMISRTPEVTCVVVDVSHEDPEVKFNWYVDGVEVHNAKTKPREEQYNSTYRVVSVLTVLHQDWLNGKEYKCKVSNKALPAPIEKTISKAKGQPREPQVYTLPPSRDELTKNQVSLTCLVKGFYPSDIAVEWESNGQPENNYRTTPPVLLSDGSFFLYSRLTVDKSRWQQGNVFSCSVMHEALHNHYTQKSLSLSPGK

SEQ ID NO: 81 - protein, 223 aa, Artificial Sequence
  B215 Fc (CH3B included)
TCPPCPAPELLGGPSVFLFPPKPKDTLMISRTPEVTCVVVDVSHEDPEVKFNWYVDGVEVHNAKTKPREEQYNSTYRVVSVLTVLHQDWLNGKEYKCKVSNKALPAPIEKTISKAKGQPREPQVYTLPPSRDELTKNQVSLTCLVKGFYPSDIAVEWESNGQPENNYGTTPPVLWSDGSFFLYSMLTVDKSRWQQGNVFSCSVMHEALHNHYTQKSLSLSPGK

SEQ ID NO: 82 - protein, 223 aa, Artificial Sequence
  B235 Fc (CH3A included)
TCPPCPAPELLGGPSVFLFPPKPKDTLMISRTPEVTCVVVDVSHEDPEVKFNWYVDGVEVHNAKTKPREEQYNSTYRVVSVLTVLHQDWLNGKEYKCKVSNKALPAPIEKTISKAKGQPREPQVYTLPPSRDELTKNQVSLTCLVKGFYPSDIAVEWESNGQPENNYCTTPPVLLSDGSFFLYSKLTVDKSRWQQGNVFSCSVMHEALHNHYTQKSLSLSPGK

SEQ ID NO: 83 - protein, 223 aa, Artificial Sequence
  B235 Fc (CH3B included)
TCPPCPAPELLGGPSVFLFPPKPKDTLMISRTPEVTCVVVDVSHEDPEVKFNWYVDGVEVHNAKTKPREEQYNSTYRVVSVLTVLHQDWLNGKEYKCKVSNKALPAPIEKTISKAKGQPREPQVYTLPPSRDELTKNQVSLTCLVKGFYPSDIAVEWESNGQPENNYGTTPPVLCSDGSFFLYSMLTVDKSRWQQGNVFSCSVMHEALHNHYTQKSLSLSPGK

SEQ ID NO: 84 - protein, 223 aa, Artificial Sequence; identical to SEQ ID NO: 34
  B239 Fc (CH3A included)

SEQ ID NO: 85 - protein, 223 aa, Artificial Sequence; identical to SEQ ID NO: 35
  B239 Fc (CH3B included)

SEQ ID NO: 86 - protein, 223 aa, Artificial Sequence
  B240 Fc (CH3A included)
TCPPCPAPELLGGPSVFLFPPKPKDTLMISRTPEVTCVVVDVSHEDPEVKFNWYVDGVEVHNAKTKPREEQYNSTYRVVSVLTVLHQDWLNGKEYKCKVSNKALPAPIEKTISKAKGQPREPQVYTLPPSRDELTKNQVSLTCLVKGFYPSDIAVEWESNGQPENNYSTTPPVLLSDGSFFLYSRLTVDKSRWQQGNVFSCSVMHEALHNHYTQKSLSLSPGK

SEQ ID NO: 87 - protein, 223 aa, Artificial Sequence; identical to SEQ ID NO: 79
  B240 Fc (CH3B included)

SEQ ID NO: 88 - protein, 223 aa, Artificial Sequence
  B256 Fc (CH3A included)
TCPPCPAPELLGGPSVFLFPPKPKDTLMISRTPEVTCVVVDVSHEDPEVKFNWYVDGVEVHNAKTKPREEQYNSTYRVVSVLTVLHQDWLNGKEYKCKVSNKALPAPIEKTISKAKGQPREPQVYTLPPSRDELTKNQVSLTCLVKGFYPSDIAVEWESNGQPENNYNTTPPVLLSDGSFFLYSKLTVDKSRWQQGNVFSCSVMHEALHNHYTQKSLSLSPGK

SEQ ID NO: 89 - protein, 223 aa, Artificial Sequence
  B256 Fc (CH3B included)
TCPPCPAPELLGGPSVFLFPPKPKDTLMISRTPEVTCVVVDVSHEDPEVKFNWYVDGVEVHNAKTKPREEQYNSTYRVVSVLTVLHQDWLNGKEYKCKVSNKALPAPIEKTISKAKGQPREPQVYTLPPSRDELTKNQVSLTCLVKGFYPSDIAVEWESNGQPENNYGTTPPVLVSDGSFFLYSMLTVDKSRWQQGNVFSCSVMHEALHNHYTQKSLSLSPGK

SEQ ID NO: 90 - protein, 223 aa, Artificial Sequence
  A107w/oW-VT Fc (CH3A included)
TCPPCPAPELLGGPSVFLFPPKPKDTLMISRTPEVTCVVVDVSHEDPEVKFNWYVDGVEVHNAKTKPREEQYNSTYRVVSVLTVLHQDWLNGKEYKCKVSNKALPAPIEKTISKAKGQPREPQVYTLPPSRDELTKNQVSLTCLVEGFYPSDIAVEWESNGQPENNYKTTPPVLDSDGSFFLYSKLTVDKSRWQQGNVFSCSVMHEALHNHYTQKSLSLSPGK

SEQ ID NO: 91 - protein, 223 aa, Artificial Sequence; identical to SEQ ID NO: 75
  A107w/oW-VT Fc (CH3B included)

SEQ ID NO: 92 - protein, 223 aa, Artificial Sequence
  A109w/oW-VT Fc (CH3A included)
TCPPCPAPELLGGPSVFLFPPKPKDTLMISRTPEVTCVVVDVSHEDPEVKFNWYVDGVEVHNAKTKPREEQYNSTYRVVSVLTVLHQDWLNGKEYKCKVSNKALPAPIEKTISKAKGQPREPQVYTLPPSRDELTKNQVSLTCLVMGFYPSDIAVEWESNGQPENNYKTTPPVLDSDGSFFLYSKLTVDKSRWQQGNVFSCSVMHEALHNHYTQKSLSLSPGK

SEQ ID NO: 93 - protein, 223 aa, Artificial Sequence
  A109w/oW-VT Fc (CH3B included)
TCPPCPAPELLGGPSVFLFPPKPKDTLMISRTPEVTCVVVDVSHEDPEVKFNWYVDGVEVHNAKTKPREEQYNSTYRVVSVLTVLHQDWLNGKEYKCKVSNKALPAPIEKTISKAKGQPREPQVYTLPPSRDMLTKNQVWLTCLVKGFYPSDIAVEWESNGQPENNYKTTPPVLDSDGSFFLYSKLTVDKSRWQQGNVFSCSVMHEALHNHYTQKSLSLSPGK

SEQ ID NO: 94 - protein, 223 aa, Artificial Sequence
  A146w/oW-VT Fc (CH3A included)
TCPPCPAPELLGGPSVFLFPPKPKDTLMISRTPEVTCVVVDVSHEDPEVKFNWYVDGVEVHNAKTKPREEQYNSTYRVVSVLTVLHQDWLNGKEYKCKVSNKALPAPIEKTISKAKGQPREPQVYTLPPSRDELTKNQVSLTCLVDGFYPSDIAVEWESNGQPENNYKTTPPVLDSDGSFFLYSKLTVDKSRWQQGNVFSCSVMHEALHNHYTQKSLSLSPGK

SEQ ID NO: 95 - protein, 223 aa, Artificial Sequence
  A146w/oW-VT Fc (CH3B included)
TCPPCPAPELLGGPSVFLFPPKPKDTLMISRTPEVTCVVVDVSHEDPEVKFNWYVDGVEVHNAKTKPREEQYNSTYRVVSVLTVLHQDWLNGKEYKCKVSNKALPAPIEKTISKAKGQPREPQVYTLPPSRDMLTKNQVSLTCLVKGFYPSDIAVEWESNGQPENNYKTTPPVLDSDGSFFLYSKLTVDKSRWQQGNVFSCSVMHEALHNHYTQKSLSLSPGK

SEQ ID NO: 96 - protein, 223 aa, Artificial Sequence
  B168w/oW-VT Fc (CH3A included)
TCPPCPAPELLGGPSVFLFPPKPKDTLMISRTPEVTCVVVDVSHEDPEVKFNWYVDGVEVHNAKTKPREEQYNSTYRVVSVLTVLHQDWLNGKEYKCKVSNKALPAPIEKTISKAKGQPREPQVYTLPPSRDELTKNQVSLTCLVKGFYPSDIAVEWESNGQPENNYKTTPPVLLSDGSFFLYSKLTVDKSRWQQGNVFSCSVMHEALHNHYTQKSLSLSPGK

SEQ ID NO: 97 - protein, 223 aa, Artificial Sequence
  B168w/oW-VT Fc (CH3B included)
TCPPCPAPELLGGPSVFLFPPKPKDTLMISRTPEVTCVVVDVSHEDPEVKFNWYVDGVEVHNAKTKPREEQYNSTYRVVSVLTVLHQDWLNGKEYKCKVSNKALPAPIEKTISKAKGQPREPQVYTLPPSRDELTKNQVSLTCLVKGFYPSDIAVEWESNGQPENNYGTTPPVLDSDGSFFLYSMLTVDKSRWQQGNVFSCSVMHEALHNHYTQKSLSLSPGK

SEQ ID NO: 98 - protein, 223 aa, Artificial Sequence
  KiH (Genentech) Fc (CH3A included)
TCPPCPAPELLGGPSVFLFPPKPKDTLMISRTPEVTCVVVDVSHEDPEVKFNWYVDGVEVHNAKTKPREEQYNSTYRVVSVLTVLHQDWLNGKEYKCKVSNKALPAPIEKTISKAKGQPREPQVYTLPPSRDELTKNQVSLSCAVKGFYPSDIAVEWESNGQPENNYKTTPPVLDSDGSFFLVSKLTVDKSRWQQGNVFSCSVMHEALHNHYTQKSLSLSPGK

SEQ ID NO: 99 - protein, 223 aa, Artificial Sequence
  KiH (Genentech) Fc (CH3B included)
TCPPCPAPELLGGPSVFLFPPKPKDTLMISRTPEVTCVVVDVSHEDPEVKFNWYVDGVEVHNAKTKPREEQYNSTYRVVSVLTVLHQDWLNGKEYKCKVSNKALPAPIEKTISKAKGQPREPQVYTLPPSRDELTKNQVSLWCLVKGFYPSDIAVEWESNGQPENNYKTTPPVLDSDGSFFLYSKLTVDKSRWQQGNVFSCSVMHEALHNHYTQKSLSLSPGK

SEQ ID NO: 100 - protein, 223 aa, Artificial Sequence; identical to SEQ ID NO: 98
  Hole-Hole (Genentech) Fc (CH3A included)